European Patent Application EP 4 545 090 A1, published April 30, 2025. Title: TF-IFNAR1. Applicant: Universität Leipzip. The sequence listing filed with the application follows.

SEQUENCE LISTING (2 sequences)

SEQ ID NO: 1 - protein, 295 aa, human [sequence omitted]

SEQ ID NO: 2 - protein, 387 aa, human
MMVVLLGATTLVLVAVAPWVLSAAAGGKNLKSPQKVEVDIIDDNFILRWNRSDESVGNVTFSFDYQKTGMDNWIKLSGCQNITSTKCNFSSLKLNVYEEIKLRIRAEKENTSSWYEVDSFTPFRKAQIGPPEVHLEAEDKAIVIHISPGTKDSVMWALDGLSFTYSLVIWKNSSGVEERIENIYSRHKIYKLSPETTYCLKVKAALLTSWKIGVYSPVHCIKTTVENELPPPENIEVSVQNQNYVLKWDYTYANMTFQVQWLHAFLKRNPGNHLYKWKQIPDCENVKTTQCVFPQNVFQKGIYLLRVQASDGNNTSFWSEEIKFDTEIQAFLLPPVFNIRSLSDSFHIYIGAPKQSGNTPVIQDYPLIYEIIFWENTSNAERKKKKK